European Patent Application EP 4 148 146 A1, published March 15, 2023. Title: Method to generate personalized neoantigens of a tumor of a patient. Applicant: OncoDNA. The sequence listing filed with the application follows.

SEQUENCE LISTING (60 sequences)

SEQ ID NO: 1 - protein, 27 aa, Artificial Sequence
  Neoantigen amino acid sequence of SEQ ID NO :1 (F01OncoRNA1)
PRLVPGWTKPITIGSHAHGDQVGQGGE

SEQ ID NO: 2 - protein, 27 aa, artificial sequence
  Neoantigen amino acid sequence of SEQ ID NO :2 (F02OncoRNA1)
EAALFGRFTIKSDVWSFRILLTELITK

SEQ ID NO: 3 - protein, 27 aa, artificial sequence
  Neoantigen amino acid sequence of SEQ ID NO :3 (F03OncoRNA1)
IDFVLSNARPVLGVGGAAMLGIATLAV

SEQ ID NO: 4 - protein, 27 aa, artificial sequence
  Neoantigen amino acid sequence of SEQ ID NO :4 (F040ncoRNA1)
RQHRDRDREKEREKEKGKPKPRSPQPL

SEQ ID NO: 5 - protein, 27 aa, artificial sequence
  Neoantigen amino acid sequence of SEQ ID NO :5 (F050ncoRNA1)
KQQEVQFKSYYLPKDDEYYQFCYVDED

SEQ ID NO: 6 - protein, 27 aa, artificial sequence
  Neoantigen amino acid sequence of SEQ ID NO :6 (F06OncoRNA1)
VVYFTAMFPYVVLVILLIRGVTLPGAG

SEQ ID NO: 7 - protein, 27 aa, artificial sequence
  Neoantigen amino acid sequence of SEQ ID NO :7 (F07OncoRNA1)
AGDAPTFPRPSGPRNTLWQELPAVQAS

SEQ ID NO: 8 - protein, 27 aa, artificial sequence
  Neoantigen amino acid sequence of SEQ ID NO :8 (F08OncoRNA1)
HNLIAEVGAPAALGVRGALEGLPRPPP

SEQ ID NO: 9 - protein, 27 aa, artificial sequence
  Neoantigen amino acid sequence of SEQ ID NO :9 (F09OncoRNA1)
NIPRLVPGWTKPITIGSHAHGDQVGQG

SEQ ID NO: 10 - protein, 27 aa, artificial sequence
  Neoantigen amino acid sequence of SEQ ID NO :10 (F10OncoRNA1)
CLQDWGPFFSLAVPSMLMICFEWWAYE

SEQ ID NO: 11 - protein, 27 aa, artificial sequence
  Neoantigen amino acid sequence of SEQ ID NO :11 (F11OncoRNA1)
FVLSNARPVLGVGGAAMLGIATLAVKR

SEQ ID NO: 12 - protein, 27 aa, artificial sequence
  Neoantigen amino acid sequence of SEQ ID NO :12 (F12OncoRNA1)
AITRAESFSVMYAPFATKIRADKIEKV

SEQ ID NO: 13 - protein, 27 aa, artificial sequence
  Neoantigen amino acid sequence of SEQ ID NO :13 (F13OncoRNA1)
GWKTTCEYYTFMWVTLPIDLNNKSAKQ

SEQ ID NO: 14 - protein, 27 aa, artificial sequence
  Neoantigen amino acid sequence of SEQ ID NO :14 (F14OncoRNA1)
WEEFTDQLSFIGRIRPLAEKTGICKIR

SEQ ID NO: 15 - protein, 27 aa, artificial sequence
  Neoantigen amino acid sequence of SEQ ID NO :15 (F15OncoRNA1)
LPGIGHACGHNLIAEVGAPAALGVRGA

SEQ ID NO: 16 - protein, 27 aa, artificial sequence
  Neoantigen amino acid sequence of SEQ ID NO :16 (F16OncoRNA1)
FSEDGEYFAYGVSASGSDWVTIKFMKV

SEQ ID NO: 17 - protein, 27 aa, artificial sequence
  Neoantigen amino acid sequence of SEQ ID NO :17 (F17OncoRNA1)
CGGGIQTREVYCAQSLPAAAALRAKEV

SEQ ID NO: 18 - protein, 27 aa, artificial sequence
  Neoantigen amino acid sequence of SEQ ID NO :18 (F18OncoRNA1)
PDAMLLAEIRSVGQTEYNGFHLSKKIV

SEQ ID NO: 19 - protein, 27 aa, artificial sequence
  Neoantigen amino acid sequence of SEQ ID NO :19 (F19OncoRNA1)
SSGKLLAKTVYLREAEGMFDIHIVQNP

SEQ ID NO: 20 - protein, 27 aa, artificial sequence
  Neoantigen amino acid sequence of SEQ ID NO :20 (F20OncoRNA1)
SVPGAVLMDIKSELLRYEIQFKGNAHT

SEQ ID NO: 21 - protein, 27 aa, artificial sequence
  Neoantigen amino acid sequence of SEQ ID NO :21 (F21OncoRNA1)
SKQEGFIDTALRKYVENLVLHGIPMAS

SEQ ID NO: 22 - protein, 27 aa, artificial sequence
  Neoantigen amino acid sequence of SEQ ID NO :22 (F22OncoRNA1)
IMNHADSATGKVKIEREGVFYPLLLQS

SEQ ID NO: 23 - protein, 27 aa, artificial sequence
  Neoantigen amino acid sequence of SEQ ID NO :23 (F23OncoRNA1)
ASPSNLKGKTEIFAHVELRVMQGLYID

SEQ ID NO: 24 - protein, 27 aa, artificial sequence
  Neoantigen amino acid sequence of SEQ ID NO :24 (F24OncoRNA1)
EAGVGFLSKDRKIALYLTNEHQVSMPI

SEQ ID NO: 25 - protein, 27 aa, artificial sequence
  Neoantigen amino acid sequence of SEQ ID NO :25 (F25OncoRNA1)
SMLRFYNKGVKGPLEASDTVEHALIQI

SEQ ID NO: 26 - protein, 27 aa, artificial sequence
  Neoantigen amino acid sequence of SEQ ID NO :26 (F26OncoRNA1)
VFPLEEQMGKITRDGSYHIAVLANSKL

SEQ ID NO: 27 - protein, 27 aa, artificial sequence
  Neoantigen amino acid sequence of SEQ ID NO :27 (F27OncoRNA1)
SELYKRAGKMNTVGLSQEAILIDPFHV

SEQ ID NO: 28 - protein, 27 aa, artificial sequence
  Neoantigen amino acid sequence of SEQ ID NO :28 (F28OncoRNA1)
SLLGLKQISPVDRAAMEIYNVFHGKTE

SEQ ID NO: 29 - protein, 27 aa, artificial sequence
  Neoantigen amino acid sequence of SEQ ID NO :29 (F29OncoRNA1)
IVTAGRPHLLEMLNSVQFAGESKYKID

SEQ ID NO: 30 - protein, 27 aa, artificial sequence
  Neoantigen amino acid sequence of SEQ ID NO :30 (F30OncoRNA1)
VAHGSEQTEIPFYSGLVNIDLAKLKRM

SEQ ID NO: 31 - protein, 27 aa, artificial sequence
  Neoantigen amino acid sequence of SEQ ID NO :31 (F31OncoRNA1)
QYLSPMVHILGLERVAKNTEKFAGISD

SEQ ID NO: 32 - protein, 27 aa, artificial sequence
  Neoantigen amino acid sequence of SEQ ID NO :32 (F32OncoRNA1)
MSQVIEIKNRALAGHFTDYLEGVSKPL

SEQ ID NO: 33 - protein, 27 aa, artificial sequence
  Neoantigen amino acid sequence of SEQ ID NO :33 (F33OncoRNA1)
MLAISLRGYPSGAVHINTEVEQKLKDF

SEQ ID NO: 34 - protein, 27 aa, artificial sequence
  Neoantigen amino acid sequence of SEQ ID NO :34 (F34OncoRNA1)
VEPLSLFKKNLGYRTIQHAMADSEVIG

SEQ ID NO: 35 - protein, 27 aa, artificial sequence
  Neoantigen amino acid sequence of SEQ ID NO :35 (F35OncoRNA1)
SKVKVLNISELHGYEFQAMGTRDPAIL

SEQ ID NO: 36 - protein, 27 aa, artificial sequence
  Neoantigen amino acid sequence of SEQ ID NO :36 (F36OncoRNA1)
HKKLALIGPNQDVRMTLSGFEASVEIY

SEQ ID NO: 37 - protein, 27 aa, artificial sequence
  Neoantigen amino acid sequence of SEQ ID NO :37 (F37OncoRNA1)
PGHASFVMAYIQERLKVNTKLLDGISE

SEQ ID NO: 38 - protein, 27 aa, artificial sequence
  Neoantigen amino acid sequence of SEQ ID NO :38 (F38OncoRNA1)
KDVIESVKALSINRYTLFGAQMHEPLG

SEQ ID NO: 39 - protein, 27 aa, artificial sequence
  Neoantigen amino acid sequence of SEQ ID NO :39 (F39OncoRNA1)
QHVRAIKKFEILMYSSGNTPVEGALLD

SEQ ID NO: 40 - protein, 27 aa, artificial sequence
  Neoantigen amino acid sequence of SEQ ID NO :40 (F40OncoRNA1)
GVSTDRIKMEQYLLFESNGKHLVIPAA

SEQ ID NO: 41 - protein, 27 aa, artificial sequence
  Neoantigen amino acid sequence of SEQ ID NO :41 (F41OncoRNA1)
TIKDYSRSHLKGMPLFAVIVLEQENAG

SEQ ID NO: 42 - protein, 27 aa, artificial sequence
  Neoantigen amino acid sequence of SEQ ID NO :42 (F42OncoRNA1)
MIEQDVAEIGLRLAYKVSSPTLHFNGK

SEQ ID NO: 43 - protein, 27 aa, artificial sequence
  Neoantigen amino acid sequence of SEQ ID NO :43 (F43OncoRNA1)
YKLQRHIDKEGTNLGFMVALPESVIAS

SEQ ID NO: 44 - protein, 27 aa, artificial sequence
  Neoantigen amino acid sequence of SEQ ID NO :44 (F44OncoRNA1)
IMHAVQKTLILREPKNDLSYGEGSAVF

SEQ ID NO: 45 - protein, 27 aa, artificial sequence
  Neoantigen amino acid sequence of SEQ ID NO :45 (F45OncoRNA1)
KAPAENMTKYSGHRGVSELFQDVLILI

SEQ ID NO: 46 - protein, 27 aa, artificial sequence
  Neoantigen amino acid sequence of SEQ ID NO :46 (F46OncoRNA1)
AVSHLGERYQGTAKIMSPLLFNKDVEI

SEQ ID NO: 47 - protein, 27 aa, artificial sequence
  Neoantigen amino acid sequence of SEQ ID NO :47 (F47OncoRNA1)
EPALDTLEYMSLHKGKNVFQSAGIRVI

SEQ ID NO: 48 - protein, 27 aa, artificial sequence
  Neoantigen amino acid sequence of SEQ ID NO :48 (F48OncoRNA1)
FDMNKKLIHQYETPSAGIRLVVEGSAL

SEQ ID NO: 49 - protein, 27 aa, artificial sequence
  Neoantigen amino acid sequence of SEQ ID NO :49 (F49OncoRNA1)
VNEQVSLRGSYFTAKAHMLDIIELGPK

SEQ ID NO: 50 - protein, 27 aa, artificial sequence
  Neoantigen amino acid sequence of SEQ ID NO :50 (F50OncoRNA1)
LPQLGKIFGRMNTKADALSEIEVYHSV

SEQ ID NO: 51 - protein, 27 aa, artificial sequence
  Neoantigen amino acid sequence of SEQ ID NO :51 (F51OncoRNA1)
KDRAEASKIPHLLLVMGEFITQYNVGS

SEQ ID NO: 52 - protein, 27 aa, artificial sequence
  Neoantigen amino acid sequence of SEQ ID NO :52 (F52OncoRNA1)
EGVFEMKRKGIQALNASDPHYILVLTS

SEQ ID NO: 53 - protein, 27 aa, artificial sequence
  Neoantigen amino acid sequence of SEQ ID NO :53 (F53OncoRNA1)
MKLGKVHEQSPLINLITASRFAGDYVE

SEQ ID NO: 54 - protein, 27 aa, artificial sequence
  Neoantigen amino acid sequence of SEQ ID NO :54 (F54OncoRNA1)
LLHIGDLKKMNFQARGAVEYSTSVIEP

SEQ ID NO: 55 - protein, 27 aa, artificial sequence
  Neoantigen amino acid sequence of SEQ ID NO :55 (F55OncoRNA1)
KHFRIPVANTGGDVLLSEKMSAYELIQ

SEQ ID NO: 56 - protein, 27 aa, artificial sequence
  Neoantigen amino acid sequence of SEQ ID NO :56 (F56OncoRNA1)
LYKMRKLDEAELFIGGITNPSAVHVQS

SEQ ID NO: 57 - protein, 27 aa, artificial sequence
  Neoantigen amino acid sequence of SEQ ID NO :57 (F57OncoRNA1)
LNIVYPQMRKIEDAKTSLSEAFLGGHV

SEQ ID NO: 58 - protein, 27 aa, artificial sequence
  Neoantigen amino acid sequence of SEQ ID NO :58 (F58OncoRNA1)
GKEEIILSSDNGYAFKRLHMPQLVTVA

SEQ ID NO: 59 - protein, 27 aa, artificial sequence
  Neoantigen amino acid sequence of SEQ ID NO :59 (F59OncoRNA1)
DFSEGGLYNAQKEKPLAVILHRVMSTI

SEQ ID NO: 60 - protein, 27 aa, artificial sequence
  Neoantigen amino acid sequence of SEQ ID NO :60 (F60OncoRNA1)
SHAKEVATGSLIQFRLGEPMDIYKVLN